European Patent Application EP 4 595 978 A1, published August 6, 2025. Title: ANTI-CD33 ANTIBODY AND ANTI-CD33 ANTIBODY-DRUG CONJUGATE AND USE THEREOF. Applicant: Systimmune, Inc. Application EP 23870708.7, filed September 25, 2023. The sequence listing filed with the application follows.

SEQUENCE LISTING (28 sequences)

SEQ ID NO: 1 - protein, 116 aa, synthetic construct [sequence omitted]

SEQ ID NO: 2 - protein, 5 aa, synthetic construct
DSNIH

SEQ ID NO: 3 - protein, 17 aa, synthetic construct
YIYPYNGGTDYNQKFKN

SEQ ID NO: 4 - protein, 7 aa, synthetic construct
GNPWLAY

SEQ ID NO: 5 - protein, 445 aa, synthetic construct
EVQLVQSGAEVKKPGSSVKVSCKASGYTITDSNIHWVRQAPGQSLEWIGYIYPYNGGTDYNQKFKNRATLTVDNPTNTAYMELSSLRSEDTAFYYCVNGNPWLAYWGQGTLVTVSSASTKGPSVFPLAPSSKSTSGGTAALGCLVKDYFPEPVTVSWNSGALTSGVHTFPAVLQSSGLYSLSSVVTVPSSSLGTQTYICNVNHKPSNTKVDKRVEPKSCDKTHTCPPCPAPELLGGPSVFLFPPKPKDTLMISRTPEVTCVVVDVSHEDPEVKFNWYVDGVEVHNAKTKPREEQYNSTYRVVSVLTVLHQDWLNGKEYKCKVSNKALPAPIEKTISKAKGQPREPQVYTLPPSRDELTKNQVSLTCLVKGFYPSDIAVEWESNGQPENNYKTTPPVLDSDGSFFLYSKLTVDKSRWQQGNVFSCSVMHEALHNHYTQKSLSLSPG

SEQ ID NO: 6 - protein, 329 aa, synthetic construct
ASTKGPSVFPLAPSSKSTSGGTAALGCLVKDYFPEPVTVSWNSGALTSGVHTFPAVLQSSGLYSLSSVVTVPSSSLGTQTYICNVNHKPSNTKVDKRVEPKSCDKTHTCPPCPAPELLGGPSVFLFPPKPKDTLMISRTPEVTCVVVDVSHEDPEVKFNWYVDGVEVHNAKTKPREEQYNSTYRVVSVLTVLHQDWLNGKEYKCKVSNKALPAPIEKTISKAKGQPREPQVYTLPPSRDELTKNQVSLTCLVKGFYPSDIAVEWESNGQPENNYKTTPPVLDSDGSFFLYSKLTVDKSRWQQGNVFSCSVMHEALHNHYTQKSLSLSPG

SEQ ID NO: 7 - protein, 111 aa, synthetic construct [sequence omitted]

SEQ ID NO: 8 - protein, 15 aa, synthetic construct
RASESLDNYGIRFLT

SEQ ID NO: 9 - protein, 7 aa, synthetic construct
AASNQGS

SEQ ID NO: 10 - protein, 9 aa, synthetic construct
QQTKEVPWS

SEQ ID NO: 11 - protein, 218 aa, synthetic construct
DIQLTQSPSTLSASVGDRVTITCRASESLDNYGIRFLTWFQQKPGKAPKLLMYAASNQGSGVPSRFSGSGSGTEFTLTISSLQPDDFATYYCQQTKEVPWSFGQGTKVEVKRTVAAPSVFIFPPSDEQLKSGTASVVCLLNNFYPREAKVQWKVDNALQSGNSQESVTEQDSKDSTYSLSSTLTLSKADYEKHKVYACEVTHQGLSSPVTKSFNRGEC

SEQ ID NO: 12 - protein, 107 aa, synthetic construct [sequence omitted]

SEQ ID NO: 13 - DNA, 348 bp, synthetic construct
  source 1..348: mol_type = other DNA
gaggtgcagctggtgcagagtggagctgaggtgaagaagccaggctcctctgtgaaggtgtcctgcaaggcctctggctacaccatcacagacagcaacatccactgggtgaggcaggccccaggccagagcctggagtggattggctacatctacccctacaatggaggcacagactacaaccagaagttcaagaacagagccaccctgactgtggacaaccccaccaacacagcctacatggagctgagctccctgagaagtgaagacacagccttctactactgtgtgaatgggaacccctggctggcctactggggccagggcaccctggtgactgtgtcctct

SEQ ID NO: 14 - DNA, 15 bp, synthetic construct
  source 1..15: mol_type = other DNA
gacagcaacatccac

SEQ ID NO: 15 - DNA, 51 bp, synthetic construct
  source 1..51: mol_type = other DNA
tacatctacccctacaatggaggcacagactacaaccagaagttcaagaac

SEQ ID NO: 16 - DNA, 21 bp, synthetic construct
  source 1..21: mol_type = other DNA
gggaacccctggctggcctac

SEQ ID NO: 17 - DNA, 1338 bp, synthetic construct
  source 1..1338: mol_type = other DNA
gaggtgcagctggtgcagagtggagctgaggtgaagaagccaggctcctctgtgaaggtgtcctgcaaggcctctggctacaccatcacagacagcaacatccactgggtgaggcaggccccaggccagagcctggagtggattggctacatctacccctacaatggaggcacagactacaaccagaagttcaagaacagagccaccctgactgtggacaaccccaccaacacagcctacatggagctgagctccctgagaagtgaagacacagccttctactactgtgtgaatgggaacccctggctggcctactggggccagggcaccctggtgactgtgtcctctgctagcaccaagggcccctctgtgttccctctggctccctcctccaagagcacctctggaggcacagctgccctgggctgcctggtgaaggactacttcccagagcctgtgactgtgtcctggaactctggagccctgacctctggagtgcacaccttcccagctgtgctgcagagctctggcctctacagcctgtcctctgtggtgactgtgccctcctcctccctgggaacccagacctacatctgcaatgtgaaccacaagccctccaacaccaaggtggacaagagagtggagcccaagagctgtgacaagacccacacctgcccaccctgcccagccccagagctgctgggaggaccctctgtgttcctctttccacccaagcccaaggacaccctgatgatctccagaaccccagaggtgacctgtgtggtggtggatgtgtcccatgaagacccagaagtgaagttcaactggtatgtggatggagtggaagtgcacaatgccaagaccaagcccagagaagagcagtacaacagcacctacagagtggtgtctgtgctgactgtgctgcaccaggactggctgaatggcaaagagtacaagtgcaaagtgtccaacaaggccctgccagctcccattgagaagaccatctccaaggccaagggccagcccagagagcctcaggtgtacaccctgccaccatccagagatgagctgaccaagaaccaggtgtccctgacctgcctggtgaaaggcttctacccctctgacattgctgtggagtgggagagcaatggccagccagagaacaactacaagaccacaccacctgtgctggactctgatggcagcttcttcctgtacagcaagctgactgtggacaagagcagatggcagcagggcaatgtcttctcctgctctgtgatgcatgaagctctgcacaaccactacacccagaagagcctgtccctgtctccagggtga

SEQ ID NO: 18 - DNA, 990 bp, synthetic construct
  source 1..990: mol_type = other DNA
gctagcaccaagggcccctctgtgttccctctggctccctcctccaagagcacctctggaggcacagctgccctgggctgcctggtgaaggactacttcccagagcctgtgactgtgtcctggaactctggagccctgacctctggagtgcacaccttcccagctgtgctgcagagctctggcctctacagcctgtcctctgtggtgactgtgccctcctcctccctgggaacccagacctacatctgcaatgtgaaccacaagccctccaacaccaaggtggacaagagagtggagcccaagagctgtgacaagacccacacctgcccaccctgcccagccccagagctgctgggaggaccctctgtgttcctctttccacccaagcccaaggacaccctgatgatctccagaaccccagaggtgacctgtgtggtggtggatgtgtcccatgaagacccagaagtgaagttcaactggtatgtggatggagtggaagtgcacaatgccaagaccaagcccagagaagagcagtacaacagcacctacagagtggtgtctgtgctgactgtgctgcaccaggactggctgaatggcaaagagtacaagtgcaaagtgtccaacaaggccctgccagctcccattgagaagaccatctccaaggccaagggccagcccagagagcctcaggtgtacaccctgccaccatccagagatgagctgaccaagaaccaggtgtccctgacctgcctggtgaaaggcttctacccctctgacattgctgtggagtgggagagcaatggccagccagagaacaactacaagaccacaccacctgtgctggactctgatggcagcttcttcctgtacagcaagctgactgtggacaagagcagatggcagcagggcaatgtcttctcctgctctgtgatgcatgaagctctgcacaaccactacacccagaagagcctgtccctgtctccagggtga

SEQ ID NO: 19 - DNA, 333 bp, synthetic construct
  source 1..333: mol_type = other DNA
gacatccagctgacccagagcccctccaccctgtctgcctctgtgggagacagagtgaccatcacctgcagagcctctgagagcctggacaactatggcatcagattcctgacctggttccagcagaagccagggaaagcccccaagctgctgatgtatgctgcctccaaccagggcagtggagtgccctccagattctctggctctggctctggcacagagttcaccctgaccatctcctccctgcagccagatgactttgccacctactactgccagcagaccaaggaggtgccctggagctttggacagggcaccaaggtggaggtgaag

SEQ ID NO: 20 - DNA, 45 bp, synthetic construct
  source 1..45: mol_type = other DNA
agagcctctgagagcctggacaactatggcatcagattcctgacc

SEQ ID NO: 21 - DNA, 21 bp, synthetic construct
  source 1..21: mol_type = other DNA
gctgcctccaaccagggcagt

SEQ ID NO: 22 - DNA, 27 bp, synthetic construct
  source 1..27: mol_type = other DNA
cagcagaccaaggaggtgccctggagc

SEQ ID NO: 23 - DNA, 657 bp, synthetic construct
  source 1..657: mol_type = other DNA
gacatccagctgacccagagcccctccaccctgtctgcctctgtgggagacagagtgaccatcacctgcagagcctctgagagcctggacaactatggcatcagattcctgacctggttccagcagaagccagggaaagcccccaagctgctgatgtatgctgcctccaaccagggcagtggagtgccctccagattctctggctctggctctggcacagagttcaccctgaccatctcctccctgcagccagatgactttgccacctactactgccagcagaccaaggaggtgccctggagctttggacagggcaccaaggtggaggtgaagcgtacggtggctgctccctctgtgttcatcttcccaccctctgatgagcagctgaagtctggcacagcctctgtggtgtgcctgctgaacaacttctaccccagagaagccaaggtgcagtggaaagtggacaatgccctgcagagtgggaacagccaggagagtgtgacagagcaggacagcaaggacagcacctacagcctgtcctccaccctgaccctgtccaaagctgactatgagaagcacaaagtgtatgcctgtgaagtgacccaccagggcctgtcctctcctgtgaccaagagcttcaacagaggagagtgctga

SEQ ID NO: 24 - DNA, 324 bp, synthetic construct
  source 1..324: mol_type = other DNA
cgtacggtggctgctccctctgtgttcatcttcccaccctctgatgagcagctgaagtctggcacagcctctgtggtgtgcctgctgaacaacttctaccccagagaagccaaggtgcagtggaaagtggacaatgccctgcagagtgggaacagccaggagagtgtgacagagcaggacagcaaggacagcacctacagcctgtcctccaccctgaccctgtccaaagctgactatgagaagcacaaagtgtatgcctgtgaagtgacccaccagggcctgtcctctcctgtgaccaagagcttcaacagaggagagtgctga

SEQ ID NO: 25 - protein, 219 aa, synthetic construct
DIQLTQSPSTLSASVGDRVTITCRASESLDNYGIRFLTWFQQKPGKAPKLLMYAASNQGSGVPSRFSGSGSGTEFTLTISSLQPDDFATYYCQQTKEVPWSFGQGTKVEVKRTVAAPSVFIFPPSDEQLKSGTASVVCLLNNFYPREAKVQWKVDNALQSGNSQESVTEQDSKDSTYSLSSTLTLSKADYEKHKVYACEVTHQGLSSPVCTKSFNRGEC

SEQ ID NO: 26 - protein, 108 aa, synthetic construct
RTVAAPSVFIFPPSDEQLKSGTASVVCLLNNFYPREAKVQWKVDNALQSGNSQESVTEQDSKDSTYSLSSTLTLSKADYEKHKVYACEVTHQGLSSPVCTKSFNRGEC

SEQ ID NO: 27 - DNA, 660 bp, synthetic construct
  source 1..660: mol_type = other DNA
gacatccagctgacccagagcccctccaccctgtctgcctctgtgggagacagagtgaccatcacctgcagagcctctgagagcctggacaactatggcatcagattcctgacctggttccagcagaagccagggaaagcccccaagctgctgatgtatgctgcctccaaccagggcagtggagtgccctccagattctctggctctggctctggcacagagttcaccctgaccatctcctccctgcagccagatgactttgccacctactactgccagcagaccaaggaggtgccctggagctttggacagggcaccaaggtggaggtgaagcgtacggtggctgctccctctgtgttcatcttcccaccctctgatgagcagctgaagtctggcacagcctctgtggtgtgcctgctgaacaacttctaccccagagaagccaaggtgcagtggaaagtggacaatgccctgcagagtgggaacagccaggagagtgtgacagagcaggacagcaaggacagcacctacagcctgtcctccaccctgaccctgtccaaagctgactatgagaagcacaaagtgtatgcctgtgaagtgacccaccagggcctgtcctctcctgtgtgcaccaagagcttcaacagaggagagtgctga

SEQ ID NO: 28 - DNA, 327 bp, synthetic construct
  source 1..327: mol_type = other DNA
cgtacggtggctgctccctctgtgttcatcttcccaccctctgatgagcagctgaagtctggcacagcctctgtggtgtgcctgctgaacaacttctaccccagagaagccaaggtgcagtggaaagtggacaatgccctgcagagtgggaacagccaggagagtgtgacagagcaggacagcaaggacagcacctacagcctgtcctccaccctgaccctgtccaaagctgactatgagaagcacaaagtgtatgcctgtgaagtgacccaccagggcctgtcctctcctgtgtgcaccaagagcttcaacagaggagagtgctga